European Patent Application EP 4 491 745 A1, published January 15, 2025. Title: Composition for preventing or treating cancer comprising SETMAR inhibitor. Applicant: Korea Advanced Institute of Science and Technology. The sequence listing filed with the application follows.

SEQUENCE LISTING (3 sequences)

SEQ ID NO: 1 - DNA, 21 bp, Artificial Sequence
  source 1..21: mol_type = unassigned DNA
tccgactccaattacattata

SEQ ID NO: 2 - DNA, 21 bp, Artificial Sequence
  source 1..21: mol_type = unassigned DNA
ggatggcggagtttaaggaga

SEQ ID NO: 3 - DNA, 21 bp, Artificial Sequence
  source 1..21: mol_type = unassigned DNA
gctgggttccttctcatttcc